European Patent Application EP 4 717 781 A2, published April 1, 2026. Title: METHODS FOR RELIABLE NONINVASIVE PREIMPLANTATION GENETIC TESTING. Applicant: Beijing Changping Laboratory. The sequence listing filed with the application follows.

SEQUENCE LISTING (9 sequences)

SEQ ID NO: 1 - DNA, 19 bp, synthetic construct
  source 1..19: mol_type = other DNA
agatgtgtataagagacag

SEQ ID NO: 2 - DNA, 19 bp, synthetic construct
  source 1..19: mol_type = other DNA
tctacacatattctctgtc

SEQ ID NO: 3 - DNA, 15 bp, synthetic construct
  source 1..15: mol_type = other DNA
tcaggttttcctgaa

SEQ ID NO: 4 - DNA, 68 bp, synthetic construct
  source 1..68: mol_type = other DNA
  modified_base 1: mod_base = OTHER; note = phosphorylation
ctgtctcttatacacatctgaacagaatttaatacgactcactatagggagatgtgtataagagacag

SEQ ID NO: 5 - DNA, 30 bp, synthetic construct
  source 1..30: mol_type = other DNA
nnnnnnnngggagatgtgtataagagacag

SEQ ID NO: 6 - DNA, 15 bp, synthetic construct
  source 1..15: mol_type = other DNA
agatgtgtataagag

SEQ ID NO: 7 - DNA, 25 bp, synthetic construct
  source 1..25: mol_type = other DNA
agatgtgtataagagacagtctaca

SEQ ID NO: 8-9 - skipped (2 entries)